European Patent Application EP 4 653 542 A1, published November 26, 2025. Title: Label, marker and method for analysing a biological sample. Applicant: Leica Microsystems CMS GmbH. The sequence listing filed with the application follows.

SEQUENCE LISTING (4 sequences)

SEQ ID NO: 1 - DNA, 71 bp, Synthetic construct
  source 1..71: mol_type = other DNA
aataattaaatttaaaattttaaaaatttttcccccccccaaaaatttttaaaattttaaatttaattatt

SEQ ID NO: 2 - DNA, 18 bp, Synthetic construct
  source 1..18: mol_type = other DNA
agtaggacgacatagcac

SEQ ID NO: 3 - DNA, 33 bp, Synthetic construct
  source 1..33: mol_type = other DNA
ttattaatttaaattttaaaatttttaaaaatt

SEQ ID NO: 4 - DNA, 33 bp, Synthetic construct
  source 1..33: mol_type = other DNA
aataattaaatttaaaattttaaaaatttttaa